European Patent Specification EP 3 394 097 B1, published November 26, 2025. Title: SECONDARY ANTIBODIES AGAINST IMMUNOCOMPLEXES COMPRISING CYANOBACTERIAL CYCLIC PEPTIDE HEPATOTOXINS. Applicant: Turun yliopisto. The sequence listing filed with the application follows.

SEQUENCE LISTING (54 sequences)

SEQ ID NO: 1 - protein, 20 aa, Artificial Sequence
  Peptide linker
GGGGSGAGGSGGGGTGGGGS

SEQ ID NO: 2 - protein, 12 aa, Artificial Sequence
  LCDR1
  MISC_FEATURE (10)..(10): Xaa is N, A, or Y
RASQSVSSSXLA

SEQ ID NO: 3 - protein, 7 aa, Artificial Sequence
  LCDR2
GASSRAT

SEQ ID NO: 4 - protein, 9 aa, Artificial Sequence
  LCDR3
  MISC_FEATURE (3)..(3): Xaa is Y, S, or M
  MISC_FEATURE (4)..(4): Xaa is S, Y, or H
  MISC_FEATURE (6)..(6): Xaa is T, Y, L
QQXXSXPWT

SEQ ID NO: 5 - protein, 110 aa, Artificial Sequence
  Clone SA51D1
  DOMAIN (24)..(35): CDR1
  DOMAIN (51)..(57): CDR2
  DOMAIN (90)..(98): CDR3
EIVLTQSPGTLSLSPGERATLSCRASQSVSSSNLAWYQQKPGQAPRLLIYGASSRATGVPDRFSGSGSGTDFTLTISRLEPEDFAVYYCQQMHSTPWTFGQGTKVEIKRT

SEQ ID NO: 6 - protein, 110 aa, Artificial Sequence
  Clone SA51F6
  DOMAIN (24)..(35): CDR1
  DOMAIN (51)..(57): CDR2
  DOMAIN (90)..(98): CDR3
EIVLTQSPGTLSLSPGERATLSCRASQSVSSSYLAWYQQKPGQAPRLLIYGASSRATGVPDRFSGSGSGTDFTLTISRLEPEDFAVYYCQQSSSTPWTFGQGTKVEIKRT

SEQ ID NO: 7 - protein, 110 aa, Artificial Sequence
  Clone SA56B8
  DOMAIN (24)..(35): CDR1
  DOMAIN (51)..(57): CDR2
  DOMAIN (90)..(98): CDR3
EIVLTQSPGTLSLSPGERATLSCRASQSVSSSYLAWYQQKPGQAPRLLIYGASSRATGVPDRFSGSGSGTDFTLTISRLEPEDFAVYYCQQSSSYPWTFGQGTKVEIKRT

SEQ ID NO: 8 - protein, 110 aa, Artificial Sequence
  Clone SA59G2
  DOMAIN (24)..(35): CDR1
  DOMAIN (51)..(57): CDR2
  DOMAIN (90)..(98): CDR3
EIVLTQSPGTLSLSPGERATLSCRASQSVSSSALAWYQQKPGQAPRLLIYGASSRATGVPDRFSGSGSGTDFTLTISRLEPEDFAVYYCQQSSSLPWTFGQGTKVEIKRT

SEQ ID NO: 9 - protein, 110 aa, Artificial Sequence
  Clone SA56E7
  DOMAIN (24)..(35): CDR1
  DOMAIN (51)..(57): CDR2
  DOMAIN (90)..(98): CDR3
EIVLTQSPGTLSLSPGERATLSCRASQSVSSSNLAWYQQKPGQAPRLLIYGASSRATGVPDRFSGSGSGTDFTLTISRLEPEDFAVYYCQQSYSYPWTFGQGTKVEIKRT

SEQ ID NO: 10 - protein, 109 aa, Artificial Sequence
  Clone SA51D12
  DOMAIN (24)..(35): CDR1
  DOMAIN (51)..(57): CDR2
  DOMAIN (90)..(98): CDR3
EIVLTQSPGTLSLSPGERATLSCRASQSVSSSNLAWYQQKPGQAPRLLIYGASSRATGVPDRFSGSGSGTDFTLTISRLEPEDFAVYYCQQSSTPWTFGQGTKVEIKRT

SEQ ID NO: 11 - protein, 110 aa, Artificial Sequence
  Clone SA41B5
  DOMAIN (24)..(35): CDR1
  DOMAIN (51)..(57): CDR2
  DOMAIN (90)..(98): CDR3
EIVLTQSPGTLSLSPGERATLSCRASQSVSSSNLAWYQQKPGQAPRLLIYGASSRATGVPDRFSGSGSGTDFTLTISRLEPEDFAVYYCQQSSSLPWTFGQGTKVEIKRT

SEQ ID NO: 12 - protein, 110 aa, Artificial Sequence; identical to SEQ ID NO: 11
  Clone SA32C11
  DOMAIN (24)..(35): CDR1
  DOMAIN (51)..(57): CDR2
  DOMAIN (90)..(98): CDR3

SEQ ID NO: 13 - protein, 110 aa, Artificial Sequence
  Clone SA32F1
  DOMAIN (24)..(35): CDR1
  DOMAIN (51)..(57): CDR2
  DOMAIN (90)..(98): CDR3
EIVLTQSPGTLSLSPGERATLSCRASQSVSSSALAWYQQKPGQAPRLLIYGASSRATGVPDRFSGSGSGTDFTLTISRLEPEDFAVYYCQQSSSYPWTFGQGTKVEIKRT

SEQ ID NO: 14 - protein, 110 aa, Artificial Sequence
  Clone SA34G1
  DOMAIN (24)..(35): CDR1
  DOMAIN (51)..(57): CDR2
  DOMAIN (90)..(98): CDR3
EIVLTQSPGTLSLSPGERATLSCRASQSVSSSNLAWYQQKPGQAPRLLIYGASSRATGVPDRFSGSGSGTDFTLTISRLEPEDFAVYYCQQSSSTPWTFGQGTKVEIKRT

SEQ ID NO: 15 - protein, 110 aa, Artificial Sequence
  Clone SA42E10
  DOMAIN (24)..(35): CDR1
  DOMAIN (51)..(57): CDR2
  DOMAIN (90)..(98): CDR3
EIVLTQSPGTLSLSPGERATLSCRASQSVSSSYLAWYQQKPGQAPRLLIYGASSRATGVPDRFSGSGSGTDFTLTISRLEPEDFAVYYCQQSSSLPWTFGQGTKVEIKRT

SEQ ID NO: 16 - protein, 110 aa, Artificial Sequence; identical to SEQ ID NO: 5
  Clone SA52C2
  DOMAIN (24)..(35): CDR1
  DOMAIN (51)..(57): CDR2
  DOMAIN (90)..(98): CDR3

SEQ ID NO: 17 - protein, 110 aa, Artificial Sequence
  Clone SA55D1
  DOMAIN (24)..(35): CDR1
  DOMAIN (51)..(57): CDR2
  DOMAIN (90)..(98): CDR3
EIVLTQSPGTLSLSPGERATLSCRASQSVSSSALAWYQQKPGQAPRLLIYGASSRATGVPDRFSGSGSGTDFTLTISRLEPEDFAVYYCQQSYSYPWTFGQGTKVEIKRT

SEQ ID NO: 18 - protein, 110 aa, Artificial Sequence
  Clone SA51H4
  DOMAIN (24)..(35): CDR1
  DOMAIN (51)..(57): CDR2
  DOMAIN (90)..(98): CDR3
EIVLTQSPGTLSLSPGERATLSCRASQSVSSSNLAWYQQKPGQAPRLLIYGASSRATGVPDRFSGSGSGTDFTLTISRLEPEDFAVYYCQQSSSYPWTFGQGTKVEIKRT

SEQ ID NO: 19 - protein, 110 aa, Artificial Sequence
  Clone SA41A5
  DOMAIN (24)..(35): CDR1
  DOMAIN (51)..(57): CDR2
  DOMAIN (90)..(98): CDR3
EIVLTQSPGTLSLSPGERATLSCRASQSVSSSALAWYQQKPGQAPRLLIYGASSRATGVPDRFSGSGSGTDFTLTISRLEPEDFAVYYCQQMHSTPWTFGQGTKVEIKRT

SEQ ID NO: 20 - protein, 110 aa, Artificial Sequence; identical to SEQ ID NO: 18
  Clone SA58A12
  DOMAIN (24)..(35): CDR1
  DOMAIN (51)..(57): CDR2
  DOMAIN (90)..(98): CDR3

SEQ ID NO: 21 - protein, 110 aa, Artificial Sequence; identical to SEQ ID NO: 18
  Clone SA33D5
  DOMAIN (24)..(35): CDR1
  DOMAIN (51)..(57): CDR2
  DOMAIN (90)..(98): CDR3

SEQ ID NO: 22 - protein, 110 aa, Artificial Sequence
  Clone SA41F2
  DOMAIN (24)..(35): CDR1
  DOMAIN (51)..(57): CDR2
  DOMAIN (90)..(98): CDR3
EIVLTQSPGTLSLSPGERATLSCRASQSVSSSALAWYQQKPGQAPRLLIYGASSRATGVPDRFSGSGSGTDFTLTISRLEPEDFAVYYCQQYSSTPWTFGQGTKVEIKRT

SEQ ID NO: 23 - protein, 110 aa, Artificial Sequence; identical to SEQ ID NO: 22
  Clone SA52B4
  DOMAIN (24)..(35): CDR1
  DOMAIN (51)..(57): CDR2
  DOMAIN (90)..(98): CDR3

SEQ ID NO: 24 - protein, 110 aa, Artificial Sequence
  Clone SA57D4
  DOMAIN (24)..(35): CDR1
  DOMAIN (51)..(57): CDR2
  DOMAIN (90)..(98): CDR3
EIVLTQSPGTLSLSPGERATLSCRASQSVSSSALAWYQQKPGQAPRLLIYGASSRATGVPDRFSGSGSGTDFTLTISRLEPEDFAVYYCQQSYSLPWTFGQGTKVEIKRT

SEQ ID NO: 25 - protein, 110 aa, Artificial Sequence; identical to SEQ ID NO: 18
  Clone SA56D5
  DOMAIN (24)..(35): CDR1
  DOMAIN (51)..(57): CDR2
  DOMAIN (90)..(98): CDR3

SEQ ID NO: 26 - protein, 110 aa, Artificial Sequence; identical to SEQ ID NO: 18
  Clone SA57A3
  DOMAIN (24)..(35): CDR1
  DOMAIN (51)..(57): CDR2
  DOMAIN (90)..(98): CDR3

SEQ ID NO: 27 - protein, 110 aa, Artificial Sequence; identical to SEQ ID NO: 9
  Clone SA60A1
  DOMAIN (24)..(35): CDR1
  DOMAIN (51)..(57): CDR2
  DOMAIN (90)..(98): CDR3

SEQ ID NO: 28 - protein, 110 aa, Artificial Sequence; identical to SEQ ID NO: 18
  Clone SA42A3
  DOMAIN (24)..(35): CDR1
  DOMAIN (51)..(57): CDR2
  DOMAIN (90)..(90): CDR3

SEQ ID NO: 29 - protein, 110 aa, Artificial Sequence
  Clone SA44E11
  DOMAIN (24)..(35): CDR1
  DOMAIN (51)..(57): CDR2
  DOMAIN (90)..(98): CDR3
EIVLTQSPGTLSLSPGERATLSCRASQSVSSSALAWYQQKPGQAPRLLIYGASSRATGVPDRFSGSGSGTDFTLTISRLEPEDFAVYYCQQYSSLPWTFGQGTKVEIKRT

SEQ ID NO: 30 - protein, 121 aa, Artificial Sequence
  Clone SA51D1
  DOMAIN (31)..(35): CDR1
  DOMAIN (50)..(66): CDR2
  DOMAIN (99)..(110): CDR3
EVQLLESGGGLVQPGGSLRLSCAASGFTFSNYSMHWVRQAPGKGLEWVSEITPYDGNTDYADSVKGRFTISRDNSKNTLYLQMNSLRAEDTAVYYCAREWWSSNWIYLDYWGQGTLVTVSS

SEQ ID NO: 31 - protein, 119 aa, Artificial Sequence
  Clone SA51F6
  DOMAIN (31)..(35): CDR1
  DOMAIN (50)..(66): CDR2
  DOMAIN (99)..(108): CDR3
EVQLLESGGGLVQPGGSLRLSCAASGFTFSDYWMHWVRQAPGKGLEWVSEIWYSSGYTNYADSVKGRFTISRDNSKNTLYLQMNSLRAEDTAVYYCARDAFPWDVFDYWGQGTLVTVSS

SEQ ID NO: 32 - protein, 117 aa, Artificial Sequence
  Clone SA56B8
  DOMAIN (31)..(35): CDR1
  DOMAIN (50)..(66): CDR2
  DOMAIN (99)..(106): CDR3
EVQLLESGGGLVQPGGSLRLSCAASGFTFSDYWMHWVRQAPGKGLEWVSYINPYGGYTDYADSVKGRFTISRDNSKNTLYLQMNSLRAEDTAVYYCARYVRRHFDYWGQGTLVTVSS

SEQ ID NO: 33 - protein, 120 aa, Artificial Sequence
  Clone SA59G2
  DOMAIN (31)..(35): CDR1
  DOMAIN (51)..(66): CDR2
  DOMAIN (99)..(109): CDR3
EVQLLESGGGLVQPGGSLRLSCAASGFTFSNYYMHWVRQAPGKGLEWVSYIDPVGGETYYADSVKGRFTISRDNSKNTLYLQMNSLRAEDTAVYYCARYYYWGYRAFDYWGQGTLVTVSS

SEQ ID NO: 34 - protein, 122 aa, Artificial Sequence
  Clone SA56E7
  DOMAIN (31)..(35): CDR1
  DOMAIN (50)..(66): CDR2
  DOMAIN (99)..(111): CDR3
EVQLLESGGGLVQPGGSLRLSCAASGFTFSRYYMHWVRQAPGKGLEWVSYIWPVDGETDYADSVKGRFTISRDNSKNTLYLQMNSLRAEDTAVYYCARYVYGNSVGRVFDYWGQGTLVTVSS

SEQ ID NO: 35 - protein, 122 aa, Artificial Sequence
  Clone SA51D12
  DOMAIN (31)..(35): CDR1
  DOMAIN (50)..(66): CDR2
  DOMAIN (99)..(111): CDR3
EVQLLESGGGLVQPGGSLRLSCAASGFTFSSDVMHWVRQAPGKGLEWVSVISGYDGYTRYADSVKGRFTISRDNSKNTLYLQMNSLRAEDTAVYYCARGVPYLYGAYSFDYWGQGTLVTVSS

SEQ ID NO: 36 - protein, 120 aa, Artificial Sequence
  Clone SA41B5
  DOMAIN (31)..(35): CDR1
  DOMAIN (50)..(66): CDR2
  DOMAIN (99)..(109): CDR3
EVQLLESGGGLVQPGGSLRLSCAASGFTFSSDVMHWVRQAPGKGLEWVSVINPYDGSTYYADSVKGRFTISRDNSKNTLYLQMNSLRAEDTAVYYCARAVAGQGGYFDYWGQGTLVTVSS

SEQ ID NO: 37 - protein, 119 aa, Artificial Sequence
  Clone SA32C11
  DOMAIN (31)..(35): CDR1
  DOMAIN (50)..(66): CDR2
  DOMAIN (99)..(108): CDR3
EVQLLESGGGLVQPGGSLRLSCAASGFTFSDYWMHWVRQAPGKGLEWVSEINTSNGNTYYADSVKGRFTISRDNSKNTLYLQMNSLRAEDTAVYYCARESWWPYSFDYWGQGTLVTVSS

SEQ ID NO: 38 - protein, 122 aa, Artificial Sequence
  Clone SA32F1
  DOMAIN (31)..(35): CDR1
  DOMAIN (50)..(66): CDR2
  DOMAIN (99)..(110): CDR3
EVQLLESGGGLVQPGGSLRLSCAASGFTFSNYYMHWVRQAPGKGFEWVSSIITNGGETDYADSVKGRFTISRDNSKNTLYLQMNSLRAEDTAVYYCARLPVTRPYYAVFDYWGQGTLVTVSS

SEQ ID NO: 39 - protein, 119 aa, Artificial Sequence
  Clone SA34G1
  DOMAIN (31)..(35): CDR1
  DOMAIN (50)..(66): CDR2
  DOMAIN (99)..(108): CDR3
EVQLLESGGGLVQPGGSLRLSCAASGFTFSDYWMHWVRQAPGKGLEWVSEIIPYSGYTNYADSVKGRFTISRDNSKNTLYLQMNSLRAEDTAVYYCARETWGYPSFDYWGQGTLVTVSS

SEQ ID NO: 40 - protein, 125 aa, Artificial Sequence
  Clone SA42E10
  DOMAIN (31)..(35): CDR1
  DOMAIN (50)..(66): CDR2
  DOMAIN (99)..(114): CDR3
EVQLLESGGGLVQPGGSLRLSCAASGFTFSDYAMHWVRQAPGKGLEWVSSIIPYTGTTDYADSVKGRFTISRDNSKNTLYLQMNSLRAEDTAVYYCARTDDLIGHYDVYYYFDYWGQGTLVTVSS

SEQ ID NO: 41 - protein, 118 aa, Artificial Sequence
  Clone SA52C2
  DOMAIN (31)..(35): CDR1
  DOMAIN (50)..(66): CDR2
  DOMAIN (99)..(107): CDR3
EVQLLESGGGLVQPGGSLRLSCAASGFTFSSDVMHWVRQAPGKGLEWVSEIDPSDGTTNYADSVKGRFTISRDNSKNTLYLQMNSLRAEDTAVYYCARSYLDWPLDVWGQGTLVTVSS

SEQ ID NO: 42 - protein, 121 aa, Artificial Sequence
  Clone SA55D1
  DOMAIN (31)..(35): CDR1
  DOMAIN (50)..(66): CDR2
  DOMAIN (99)..(110): CDR3
EVQLLESGGGLVQPGGSLRLSCAASGFTFSSDVMHWVRQAPGKGLEWVSVISPYDGYTRYADSVKGRFTISRDNSKNTLYLQMNSLRAEDTAVYYCARHKGGYRRAYMDYWGQGTLVTVSS

SEQ ID NO: 43 - protein, 119 aa, Artificial Sequence
  Clone SA51H4
  DOMAIN (31)..(35): CDR1
  DOMAIN (50)..(66): CDR2
  DOMAIN (99)..(108): CDR3
EVQLLESGGGLVQPGGSLRLSCAASGFTFSDYWMHWVRQAPGKGLEWVSEIWPYDGYTNYADSVKGRFTISRDNSKNTLYLQMNSLRAEDTAVYYCARDPGPEGVFDYWGQGTLVTVSS

SEQ ID NO: 44 - protein, 119 aa, Artificial Sequence
  Clone SA41A5
  DOMAIN (31)..(35): CDR1
  DOMAIN (50)..(66): CDR2
  DOMAIN (99)..(108): CDR3
EVQLLESGGGLVQPGGSLRLSCAASGFTFSNYYMHWVRQAPGKGLEWVSEINYDGETDYADSVKGRFTISRDNSKNTLYLQMNSLRAEDTAVYYCARDGFWYGTAFDYWGQGTLVTVSS

SEQ ID NO: 45 - protein, 121 aa, Artificial Sequence
  Clone SA58A12
  DOMAIN (31)..(35): CDR1
  DOMAIN (50)..(65): CDR2
  DOMAIN (98)..(110): CDR3
EVQLLESGGGLVQPGGSLRLSCAASGFTFSNYGMHWVRQAPGKGLEWVSEIWPNNGTTNYADSVKGRFTISRDNSKNTLYLQMNSLRAEDTAVYYCARESGQWWYGVFDYWGQGTLVTVSS

SEQ ID NO: 46 - protein, 123 aa, Artificial Sequence
  Clone SA33D5
  DOMAIN (31)..(35): CDR1
  DOMAIN (50)..(66): CDR2
  DOMAIN (99)..(112): CDR3
EVQLLESGGGLVQPGGSLRLSCAASGFTFSSDVMHWVRQAPGKGLEWVSEIDPNDGSTRYADSVKGRFTISRDNSKNTLYLQMNSLRAEDTAVYYCAREYGAVSWSVVVFDYWGQGTLVTVSS

SEQ ID NO: 47 - protein, 121 aa, Artificial Sequence
  Clone SA41F2
  DOMAIN (31)..(35): CDR1
  DOMAIN (50)..(66): CDR2
  DOMAIN (99)..(110): CDR3
EVQLLESGGGLVQPGGSLRLSCAASGFTFSNYGMHWVRQAPGKGLEWVSEIDYVDGNTYYADSVKGRFTISRDNSKNTLYLQMNSLRAEDTAVYYCAREVYAHGIAAFDYWGQGTLVTVSS

SEQ ID NO: 48 - protein, 121 aa, Artificial Sequence
  Clone SA52B4
  DISULFID (31)..(35): CDR1
  DISULFID (50)..(66): CDR2
  DISULFID (99)..(110): CDR3
EVQLLESGGGLVQPGGSLRLSCAASGFTFSDYSMHWVRQAPGKGLEWVSEIWTNTGYTNYADSVKGRFTISRDNSKNTLYLQMNSLRAEDTAVYYCARESWEWFSIVFDYWGQGTLVTVSS

SEQ ID NO: 49 - protein, 117 aa, Artificial Sequence
  Clone SA57D4
  DOMAIN (31)..(35): CDR1
  DOMAIN (50)..(66): CDR2
  DOMAIN (99)..(106): CDR3
EVQLLESGGGLVQPGGSLRLSCAASGFTFSGYGMHWVRQAPGKGLEWVSAISDLNGSTYYADSVKGRFTISRDNSKNTLYLQMNSLRAEDTAVYYCARNGWGDMDLWGQGTLVTVSS

SEQ ID NO: 50 - protein, 123 aa, Artificial Sequence
  Clone SA56D5
  DOMAIN (31)..(35): CDR1
  DOMAIN (50)..(66): CDR2
  DOMAIN (99)..(112): CDR3
EVQLLESGGGLVQPGGSLRLSCAASGFTFSDYYMHWVRQAPGKGLEWVSYIDGNGGYTDYADSVKGRFTISRDNSKNTLYLQMNSLRAEDTAVYYCARYWFDSSYKHRYFDYWGQGTLVTVSS

SEQ ID NO: 51 - protein, 122 aa, Artificial Sequence
  Clone SA57A3
  DOMAIN (31)..(35): CDR1
  DOMAIN (50)..(66): CDR2
  DOMAIN (99)..(111): CDR3
EVQLLESGGGLVQPGGSLRLSCAASGFTFSDYYMHWVRQAPGKGLEWVSYINTYDGNTDYADSVKGRFTISRDNSKNTLYLQMNSLRAEDTAVYYCARYYNPYTRRRVFDYWGQGTLVTVSS

SEQ ID NO: 52 - protein, 123 aa, Artificial Sequence
  Clone SA60A1
  DOMAIN (31)..(35): CDR1
  DOMAIN (50)..(66): CDR2
  DOMAIN (99)..(112): CDR3
EVQLLESGGGLVQPGGSLRLSCAASGFTFSPYYMHWVRQAPGKGLEWVSYITPYDGYTDYADSVKGRFTISRDNSKNTLYLQMNSLRAEDTAVYYCARYSYVGSVRTRVFDYWGQGTLVTVSS

SEQ ID NO: 53 - protein, 115 aa, Artificial Sequence
  Clone SA42A3
  DOMAIN (31)..(35): CDR1
  DOMAIN (50)..(66): CDR2
  DOMAIN (99)..(104): CDR3
EVQLLESGGGLVQPGGSLRLSCAASGFTFSNYSMHWVRQAPGKGLEWVSSIYYDGETDYADSVKGRFTISRDNSKNTLYLQMNSLRAEDTAVYYCARSDGDVDYWGQGTLVTVSS

SEQ ID NO: 54 - protein, 116 aa, Artificial Sequence
  Clone SA44E11
  DOMAIN (31)..(35): CDR1
  DOMAIN (50)..(66): CDR2
  DOMAIN (99)..(105): CDR3
EVQLLESGGGLVQPGGSLRLSCAASGFTFSDYYMHWVRQAPGKGLEWVSEISTYNGYTDYADSVKGRFTISRDNSKNTLYLQMNSLRAEDTAVYYCARGGEPGDDWGQGTLVTVSS